European Patent Application EP 4 617 362 A1, published September 17, 2025. Title: A method for producing a pluripotent stem cell and a method for induction of differentiation for a pluripotent stem cell. Applicant: KANEKA CORPORATION. The sequence listing filed with the application follows.

SEQUENCE LISTING (18 sequences)

SEQ ID NO: 1 - DNA, 21 bp, synthetic construct
  misc_feature 1..21: note = Synthetic DNA
  source 1..21: mol_type = other DNA
cctcatgaagatcctcaccga

SEQ ID NO: 2 - DNA, 21 bp, synthetic construct
  misc_feature 1..21: note = Synthetic DNA
  source 1..21: mol_type = other DNA
ttgccaatggtgatgacctgg

SEQ ID NO: 3 - DNA, 23 bp, synthetic construct
  misc_feature 1..23: note = Synthetic DNA
  source 1..23: mol_type = other DNA
agtgggtggaggaagctgacaac

SEQ ID NO: 4 - DNA, 24 bp, synthetic construct
  misc_feature 1..24: note = Synthetic DNA
  source 1..24: mol_type = other DNA
tcgttgtgcatagtcgctgcttga

SEQ ID NO: 5 - DNA, 22 bp, synthetic construct
  misc_feature 1..22: note = Synthetic DNA
  source 1..22: mol_type = other DNA
caccaatcccatccacactcac

SEQ ID NO: 6 - DNA, 21 bp, synthetic construct
  misc_feature 1..21: note = Synthetic DNA
  source 1..21: mol_type = other DNA
gcaaagctcctaccgtaccac

SEQ ID NO: 7 - DNA, 24 bp, synthetic construct
  misc_feature 1..24: note = Synthetic DNA
  source 1..24: mol_type = other DNA
agcctccagcagatgcaagaactc

SEQ ID NO: 8 - DNA, 24 bp, synthetic construct
  misc_feature 1..24: note = Synthetic DNA
  source 1..24: mol_type = other DNA
ttgctccacattggaaggttccca

SEQ ID NO: 9 - DNA, 23 bp, synthetic construct
  misc_feature 1..23: note = Synthetic DNA
  source 1..23: mol_type = other DNA
tcacaaagagatgatggaggaac

SEQ ID NO: 10 - DNA, 20 bp, synthetic construct
  misc_feature 1..20: note = Synthetic DNA
  source 1..20: mol_type = other DNA
acatgcaggtgagttgtcag

SEQ ID NO: 11 - DNA, 20 bp, synthetic construct
  misc_feature 1..20: note = Synthetic DNA
  source 1..20: mol_type = other DNA
atctgcacttcgtgtgcaag

SEQ ID NO: 12 - DNA, 23 bp, synthetic construct
  misc_feature 1..23: note = Synthetic DNA
  source 1..23: mol_type = other DNA
gagtctgaggatttccttagctc

SEQ ID NO: 13 - DNA, 21 bp, synthetic construct
  misc_feature 1..21: note = Synthetic DNA
  source 1..21: mol_type = other DNA
aggaatggacttgaaacaagg

SEQ ID NO: 14 - DNA, 20 bp, synthetic construct
  misc_feature 1..20: note = Synthetic DNA
  source 1..20: mol_type = other DNA
gcaaagcttgttgatcatgg

SEQ ID NO: 15 - DNA, 20 bp, synthetic construct
  misc_feature 1..20: note = Synthetic DNA
  source 1..20: mol_type = other DNA
taccaagtcgggaaggcgaa

SEQ ID NO: 16 - DNA, 20 bp, synthetic construct
  misc_feature 1..20: note = Synthetic DNA
  source 1..20: mol_type = other DNA
gggctgtccgggtgaatgta

SEQ ID NO: 17 - DNA, 23 bp, synthetic construct
  misc_feature 1..23: note = Synthetic DNA
  source 1..23: mol_type = other DNA
agcccaagtgacaagggacaact

SEQ ID NO: 18 - DNA, 24 bp, synthetic construct
  misc_feature 1..24: note = Synthetic DNA
  source 1..24: mol_type = other DNA
aaggaaccacttcgaaggtgctga